European Patent Specification EP 3 884 043 B1, published April 8, 2026. Title: Improved variants of VSV-GP. Applicant: Vira Therapeutics GmbH. The sequence listing filed with the application follows.

SEQUENCE LISTING (10 sequences)

SEQ ID NO: 1 - DNA, 1497 bp, Dandenong virus
atggggcagctcataacaatgtttgaggctttgccccacatcatcgatgaggttatcaacatagttataattgtgcttgtgataataacaagcataaaggctgtgtacaactttgctacctgtggcattattgcactgatcagcttttgcctcctagctggcagatcttgtggtttatatggtgtcaccggtcctgacatttacaaaggactctaccaattcaagtccgtggagttcaacatgtcacagctgaatttgacgatgcccaatgcatgttcagccaacaactcccaccattacatcagtatggggaagtctggcttggagctgacttttacaaatgactccatcatcagtcacaacttttgcaacctgactgatgggttcaagaaaaaaacctttgaccacacgctcatgagtatagtggcaagcctacaccttagcatcagaggaaacaccaactataaggctgtttcctgtgattttaacaatggaatcaccatccaatacaacttgtctttctctgatgcacaaagtgccatcaatcaatgcagaacttttagaggtagagttctagacatgttcaggacagctttcggagggaagtacatgaggtccggctatggttggaagggctctgatgggaaaactacttggtgcagtcagaccagttatcaatacctaatcatacagaacagaacatgggagaatcactgtgagtacgccggtccttttggcctctcaagggttctctttgctcaggaaaaaacaaaatttctcactaggagattggcagggacttttacttggacactgtcggattcctcaggaactgagaacccaggtgggtactgtctgacaaagtggatgcttatagctgctgaactcaagtgttttggaaacactgctgttgctaaatgcaatatcaatcatgatgaggaattctgtgacatgttgaggctaattgattacaacaaggctgctctgaagaaattcaaagaagacgtagagtctgcccttcatctgttcaagacaactgtgaattctctaatatctgaccagctgttaatgagaaatcatttgagggacttaatgggtgtgccctattgcaactactcgaaattctggtacttggagcatgtgaaaacaggtgatacaagtgttccaaaatgctggttggtttctaacggctcatacttaaatgaaacacatttcagtgaccagatagagcaggaagcagacaacatgatcactgagatgctcaggaaagattacatcaagaggcagggaagcactcctttggcactgatggacctattaatgttctctacatcggcatatttaatcagtgttttccttcatctgatgaaaatcccaactcatagacacattaaaggtggcacatgccctaagccacacaggttaactagtaaaggcatctgtagctgtggtgcgttcaaagtgccaggagtgaaaacagtctggaagagacgctga

SEQ ID NO: 2 - protein, 498 aa, Dandenong virus
MGQLITMFEALPHIIDEVINIVIIVLVIITSIKAVYNFATCGIIALISFCLLAGRSCGLYGVTGPDIYKGLYQFKSVEFNMSQLNLTMPNACSANNSHHYISMGKSGLELTFTNDSIISHNFCNLTDGFKKKTFDHTLMSIVASLHLSIRGNTNYKAVSCDFNNGITIQYNLSFSDAQSAINQCRTFRGRVLDMFRTAFGGKYMRSGYGWKGSDGKTTWCSQTSYQYLIIQNRTWENHCEYAGPFGLSRVLFAQEKTKFLTRRLAGTFTWTLSDSSGTENPGGYCLTKWMLIAAELKCFGNTAVAKCNINHDEEFCDMLRLIDYNKAALKKFKEDVESALHLFKTTVNSLISDQLLMRNHLRDLMGVPYCNYSKFWYLEHVKTGDTSVPKCWLVSNGSYLNETHFSDQIEQEADNMITEMLRKDYIKRQGSTPLALMDLLMFSTSAYLISVFLHLMKIPTHRHIKGGTCPKPHRLTSKGICSCGAFKVPGVKTVWKRR

SEQ ID NO: 3 - DNA, 1470 bp, Mopeia virus
atggggcagatagtcaccttctttcaagaggtgccacacatccttgaagaagtgatgaacattgtgctgatgaccctctcaatcttggccatcctaaagggcatctacaatgtgatgacctgtggaatcatcggtttgataacatttttgttcttgtgtgggagatcatgctcaagcatctataaggacaactatgagttcttctctctcgacctcgacatgtcttcactgaatgcaacgatgcctctctcctgctcaaagaacaactcccatcactacatccaagttgggaatgagacaggcctagagctgacattgacaaacactagcataattgatcataagttttgcaacctgtctgatgctcacaggaggaatctttatgacaaagcacttatgtcaatcttgacaacattccacctaagcattccagattttaaccaatatgaggcaatgtcatgtgattttaacggagggaagatctcaattcaatacaacctgtcccactcaaattatgtggatgccggcaaccactgtggcactattgcaaatggcattatggatgtttttagaagaatgtattggagcacctccctttcggttgcctctgacataagtgggactcaatgcatacagaccgattataagtatttgattattcagaacacatcatgggaggatcattgcatgttctcaagaccctcacccatgggatttttaagccttctgtcacagagaaccaggaatttctacatctcaagaagacttttgggtctttttacatggactttgagtgactcggaagggaacgacatgccaggtggttactgtctcacaaggtctatgctaatagggcttgatctgaaatgctttgggaacactgccattgcgaagtgtaatcaggcacatgatgaagaattctgtgacatgctccgcctttttgattttaataaacaagcaattagcaaactgaggtctgaagttcagcagagcataaatttgataaataaagctgtcaacgccctcatcaatgatcaactggtcatgaggaaccatttgagagatctaatgggtattccttattgcaactactctaagttttggtacttgaatgatactaggacagggagaacatccctcccaaagtgttggcttgtgaccaatgggtcatacctaaatgaaacccagttctcaacagaaattgagcaagaagccaataacatgttcactgacatgttgaggaaggagtatgagaaaaggcagagcacaacacctctggggttagtagatctttttgttttctccactagcttttatttgatctccgtgttcctccacctaatcaaaattccaacacatagacacataaaaggcaagccttgcccgaaaccacacagactcaatcacatggcaatctgttcctgtggcttctataagcaaccaggtctccccacacaatggaaaaggtga

SEQ ID NO: 4 - protein, 489 aa, Mopeia virus
MGQIVTFFQEVPHILEEVMNIVLMTLSILAILKGIYNVMTCGIIGLITFLFLCGRSCSSIYKDNYEFFSLDLDMSSLNATMPLSCSKNNSHHYIQVGNETGLELTLTNTSIIDHKFCNLSDAHRRNLYDKALMSILTTFHLSIPDFNQYEAMSCDFNGGKISIQYNLSHSNYVDAGNHCGTIANGIMDVFRRMYWSTSLSVASDISGTQCIQTDYKYLIIQNTSWEDHCMFSRPSPMGFLSLLSQRTRNFYISRRLLGLFTWTLSDSEGNDMPGGYCLTRSMLIGLDLKCFGNTAIAKCNQAHDEEFCDMLRLFDFNKQAISKLRSEVQQSINLINKAVNALINDQLVMRNHLRDLMGIPYCNYSKFWYLNDTRTGRTSLPKCWLVTNGSYLNETQFSTEIEQEANNMFTDMLRKEYEKRQSTTPLGLVDLFVFSTSFYLISVFLHLIKIPTHRHIKGKPCPKPHRLNHMAICSCGFYKQPGLPTQWKR

SEQ ID NO: 5 - DNA, 1488 bp, Ippy virus
atgggacagataataaccttctttcaggaagtgcctcacattatagaggaagtcatgaacattgttctgatcaccctatccctcttggctatcttgaagggtgtgtacaatgtcatgacttgtggtctgattggattgatttcctttctcttactgtgtgggaagtcctgctctctaatctacaaggacacatataacttctcatccattgaacttgacctctcacacctcaacatgacattgcccatgtcctgcagccgaaacaactcacaccactatgtcttcttcaacggatctggcttagagatgacattcactaacgattcacttcttaaccacaaattctgcaatctttcagacgcccataaaaagaatctttacgatcatgcgctaatgggcattgtcacaactttccacttgtcaatcccgaacttcaatcaatacgaagcaatggcctgtgacttcaatggagggaatattagcattcaatacaacttgagccacaatgatcgaacagatgcaatgaaccactgtggcactgtagctaatggtgtactggatgctttttataggttccattggggcagaaatataacctacatcgctcagttgccaaatggcgacggcactggcagatggacattctgttatgccacaagttataagtacctggttatccaaaacattagctgggctgatcattgtcaaatgtcaagaccaactcccattggctttgctagcattctgagccaacggattaggagcatttacatttcaagacgactgatgagcacattcacttggtctctatccgacagttcaggtactgagaatccaggtggctattgtctcaccagatggatgctttttgcggctgacttgaaatgctttggaaacacagccattgccaaatgtaacctgaatcatgatgaagagttctgcgacatgttgaggcttattgacttcaacaagcaagccttgaaaacattcaaatcggaggttaaccatggtctacaactaattacaaaggcgattaatgccttgatcaatgaccaactcattatgaagaatcacttaagggacctaatgggtatcccttattgcaattattcaaaattctggtatctaaatgacacaagaacaggtagagtctctctgcctaagtgctggatgatcagcaacgggacctatctaaatgagactcatttttctgatgagattgaacaggaagcagacaatatgatcacagaaatgttgagaaaagagtatcaagaaagacaagggaagaccccattgggtctagttgatctttttatttttagcacaagcttttattcaatcacagtgttcctccatctcataaagattccaacgcacagacacatcgtgggacaagggtgtcccaagccacacagactaaacagtagagcaatctgctcctgtggtgcctataaacagccgggactacccaccaagtggaagcgctga

SEQ ID NO: 6 - protein, 495 aa, Ippy virus
MGQIITFFQEVPHIIEEVMNIVLITLSLLAILKGVYNVMTCGLIGLISFLLLCGKSCSLIYKDTYNFSSIELDLSHLNMTLPMSCSRNNSHHYVFFNGSGLEMTFTNDSLLNHKFCNLSDAHKKNLYDHALMGIVTTFHLSIPNFNQYEAMACDFNGGNISIQYNLSHNDRTDAMNHCGTVANGVLDAFYRFHWGRNITYIAQLPNGDGTGRWTFCYATSYKYLVIQNISWADHCQMSRPTPIGFASILSQRIRSIYISRRLMSTFTWSLSDSSGTENPGGYCLTRWMLFAADLKCFGNTAIAKCNLNHDEEFCDMLRLIDFNKQALKTFKSEVNHGLQLITKAINALINDQLIMKNHLRDLMGIPYCNYSKFWYLNDTRTGRVSLPKCWMISNGTYLNETHFSDEIEQEADNMITEMLRKEYQERQGKTPLGLVDLFIFSTSFYSITVFLHLIKIPTHRHIVGQGCPKPHRLNSRAICSCGAYKQPGLPTKWKR

SEQ ID NO: 7 - DNA, 1548 bp, Latino virus
atgggtcaagtgattggattcttccaatcattgcccgagattattaatgaagcgttgaacattgctctgatctgtgtggctctgcttgccacaatcaagggaatggtcaacatctggaaatctggtttgatacagctcctcttcttcctcacattggcaggaagaagttgttctcattcttttacaattggaagatttcatgaatttcagagtgtgacagttaactttacacagttcatgtcctatgctccaagctcttgctcagtaaacaacacccaccattatttcaaaggtccccaaaacaccacctggggtcttgagttgactttgactaatgaatcaatgataaacatcaccaattccatgagggtcttcactaacattcatcacaatgtaaccaattgcgtgcagaacatttccgaacatgagggtgtgctcaaatggctgcttgagacaatgcacctaagcatcagcaagccaggaaaacacatcgcacctgtcatgtgtgagagacaaaaggggttgctcatcgagtacaatctcactatgaccaaagaccaccacccaaattattggaatcaagtcttgtatggactggctaaattattgggctcaagtaagcgtttgtggtttggcgcatgtaacaaggctgactgtcagatgcaatcagaccaccagcacataaaatgcaattactcgaattgcaaaggttacaccagctttaaatacttaattattcaaaataccacttgggaaaaccattgtgagtataaccatctgaacaccatccaccttctcatgagctctattggccaatcctttatcacaagaaggcttcaagcctttttaacctggacactttctgatgcactagggaatgaccttcctgggggatactgtcttgaacagtgggctgtggtgtggtttggcataaagtgttttgataacacagcaatggccaagtgcaatcagaatcatgattcagagttttgtgatatgctaaggctttttgattacaatagaaatgctattcagagcttaaatgatcaatctcaagccagattaaaccttttaactaacaccattaattcacttgtctctgacaatttactaatgaaaaataagctaagagaactaatgaacgtgccatactgtaattacactagattctggtttattaatgatacaaagaatggtagacacactcttccacaatgttggttggtatcagatggttcgtacttgaatgaaaccagattcagaactcaatggctaagtgaaagtaactctttatacacagaaatgctgactgaagaatatgaaaaaagacagggtagaacacctctttctttagtggacctatgcttttggtcaactctcttttacatatcaacattatttgcgcatttagtgggtttcccaactcacagacaccttataggtgagggctgcccaaaaccacacagattaacagggtcagggatctgctcatgtggacattatggtattccaggtaaaccagtcagatggacaaagatgtcaaggtga

SEQ ID NO: 8 - protein, 515 aa, Latino virus
MGQVIGFFQSLPEIINEALNIALICVALLATIKGMVNIWKSGLIQLLFFLTLAGRSCSHSFTIGRFHEFQSVTVNFTQFMSYAPSSCSVNNTHHYFKGPQNTTWGLELTLTNESMINITNSMRVFTNIHHNVTNCVQNISEHEGVLKWLLETMHLSISKPGKHIAPVMCERQKGLLIEYNLTMTKDHHPNYWNQVLYGLAKLLGSSKRLWFGACNKADCQMQSDHQHIKCNYSNCKGYTSFKYLIIQNTTWENHCEYNHLNTIHLLMSSIGQSFITRRLQAFLTWTLSDALGNDLPGGYCLEQWAVVWFGIKCFDNTAMAKCNQNHDSEFCDMLRLFDYNRNAIQSLNDQSQARLNLLTNTINSLVSDNLLMKNKLRELMNVPYCNYTRFWFINDTKNGRHTLPQCWLVSDGSYLNETRFRTQWLSESNSLYTEMLTEEYEKRQGRTPLSLVDLCFWSTLFYISTLFAHLVGFPTHRHLIGEGCPKPHRLTGSGICSCGHYGIPGKPVRWTKMSR

SEQ ID NO: 9 - DNA, 1557 bp, Oliveros virus
atgggtcaagtcattgggttcttccaatccttacccaacatcattaatgaggcactaaacattgccctcatctgtgtggcattaattgccatattgaaaggtattgttaacatatggaaatcaggtctgattcagctgttcatattcctcatcctagcggggaggagctgttctcacacctttcagattggccgaaaccatgagttccaaagtatcactctaaacttcacacagtttttgggctacgcacccagctcctgttctgttaacaacactcatcactactttagaggtcctggcaatgtctcttggggcatcgagctcacattgaccaacaactccgtgatcaatgcaagcaactcactgaaggtgttcaccaacattcaccacaacatcaccaactgcgttcagaatatcgatgagcaagaccacctaatgaaatggctcatagaaacaatgcatctacagatcatgaaaccaggaaagagactaccaccaatcctgtgtgagaaagacaaagggttactaattgaatacaacctaaccaacattgcatctcgcgaagaaaagcactctgagtactggagccaacttctctatggtctatcaaaactattaggctccagtaagtcattgtggtttgattactgtcagagagcagattgcatgatgcaagagcacagctcacacttgaagtgcaactactcagagtgttctggccataccaccttcaaatacctcattctacaaaacaccacttgggagaaccattgtgagttcaaccatctaaacacaattcacctgttgatgagctctactggtcagtctttcataactagaaggttgcaggcttttctaacttggactttgtcagatgctacaggcaatgacctccctgggggttactgcctagagcagtgggccatagtttgggcaggcatcaagtgctttgggaacacagcagttgcaaagtgtaatcaaaatcatgactctgaattctgtgacatgttgaggctctttgattacaataggaatgctattaagagtctgaatgatcagtctcaaagtcgtctaaatcttctaacaaatacaataaattcactgatttcggataatctgttgatgaaaaacaagttggctgagataatgaacattccgtattgcaattacacaaaattctggtacatcaacgacactaggactggaaggcacacccttccccaatgctggttaatctcaaatgggtcttacttgaatgagactaaattcagaactcagtggctgtcagagagcaatgcactctatacagaaatgctaacagaagattatgacaaaaggcagggtagcacaccactctccttggttgatctatgtttttggtcaaccttattctatgtgaccacattgtttgctcatcttgttggtttcccaacacacagacacatcttagatggtccttgccctaaaccccacagattaacaaagaaaggaatttgttcctgtggacattttggaataccgggcaaacctgttcgatgggtgaaacgatcacggtga

SEQ ID NO: 10 - protein, 518 aa, Oliveros virus
MGQVIGFFQSLPNIINEALNIALICVALIAILKGIVNIWKSGLIQLFIFLILAGRSCSHTFQIGRNHEFQSITLNFTQFLGYAPSSCSVNNTHHYFRGPGNVSWGIELTLTNNSVINASNSLKVFTNIHHNITNCVQNIDEQDHLMKWLIETMHLQIMKPGKRLPPILCEKDKGLLIEYNLTNIASREEKHSEYWSQLLYGLSKLLGSSKSLWFDYCQRADCMMQEHSSHLKCNYSECSGHTTFKYLILQNTTWENHCEFNHLNTIHLLMSSTGQSFITRRLQAFLTWTLSDATGNDLPGGYCLEQWAIVWAGIKCFGNTAVAKCNQNHDSEFCDMLRLFDYNRNAIKSLNDQSQSRLNLLTNTINSLISDNLLMKNKLAEIMNIPYCNYTKFWYINDTRTGRHTLPQCWLISNGSYLNETKFRTQWLSESNALYTEMLTEDYDKRQGSTPLSLVDLCFWSTLFYVTTLFAHLVGFPTHRHILDGPCPKPHRLTKKGICSCGHFGIPGKPVRWVKRSR